European Patent Specification EP 3 575 323 B1, published September 11, 2024. Title: ANTI-DR5 FAMILY ANTIBODIES, BISPECIFIC ANTI-DR5 FAMILY ANTIBODIES AND METHODS OF USE THEREOF. Applicant: Genmab Holding B.V. The sequence listing filed with the application follows.

SEQUENCE LISTING (41 sequences)

SEQ ID NO: 1 - DNA, 321 bp, Artificial Sequence
  Nucleic acid sequence of murine anti-DR5-01 variable light chain
gacattgtgctgacccagtctccagccaccctgtctgtgactccaggagatagcgtcagtctttcctgcagggccagccaaagtattagcaacaacctacactggtatcaacaaaaatcacatgagtctccaaggcttctcatcaagtttgcttcccagtccatctctgggatcccctcccggttcagtggcagtggatcaggggcagatttcactctcattatcaacagtgtggagactgaagattttggaatgtatttctgtcaacagggtaacagctggccgtacacattcggtggaggcaccaagctcgagatcaaa

SEQ ID NO: 2 - protein, 107 aa, Artificial Sequence
  Amino acid sequence of murine anti-DR5-01 variable light chain
DIVLTQSPATLSVTPGDSVSLSCRASQSISNNLHWYQQKSHESPRLLIKFASQSISGIPSRFSGSGSGADFTLIINSVETEDFGMYFCQQGNSWPYTFGGGTKLEIK

SEQ ID NO: 3 - DNA, 354 bp, Artificial Sequence
  Nucleic acid sequence of murine anti-DR5-01 variable heavy chain
gaggtccagctgcagcagtctggggcagagtttgtgaagccaggggcctcagtcaagttgtcctgcacagcttctggcttcaacattaaagacacctttatacactgggtgaagcagaggcctgaacagggcctggactggattggaaggattgatcctgcgaatggtaatactaaatatgatccgaagttccagggcaaggccactgaaacaacagacacatcctccaacacagcctacctgcagctcagcagcctgacatctgaggacactgccgtctattattgtgttagaggactatatacgtactactttgactactggggccaaggaacctcggtcaccgtctcctca

SEQ ID NO: 4 - protein, 118 aa, Artificial Sequence
  Amino acid sequence of murine anti-DR5-01 variable heavy chain
EVQLQQSGAEFVKPGASVKLSCTASGFNIKDTFIHWVKQRPEQGLDWIGRIDPANGNTKYDPKFQGKATETTDTSSNTAYLQLSSLTSEDTAVYYCVRGLYTYYFDYWGQGTSVTVSS

SEQ ID NO: 5 - DNA, 318 bp, Artificial Sequence
  Nucleic acid sequence of murine anti-DR5-05 variable light chain
gacattcagctgacccagtctccagcaatcatgtctgcatctccaggggagaaggtcaccatatcctgcagtgccagttcaagtgtaagttacatgtactggtaccagcagaagccaggatcctcccccaaaccctggatttatcgcacatccaacctggcttctggagtccctggtcgcttcagtggcagtgggtctgggacctcttactctctcacaatcagcagcatggaggctgaagatgctgccacttattactgccagcagtatcatagttacccacctacattcggtggaggcaccaagctcgagatcaaa

SEQ ID NO: 6 - protein, 106 aa, Artificial Sequence
  Amino acid sequence of murine anti-DR5-05 variable light chain
DIQLTQSPAIMSASPGEKVTISCSASSSVSYMYWYQQKPGSSPKPWIYRTSNLASGVPGRFSGSGSGTSYSLTISSMEAEDAATYYCQQYHSYPPTFGGGTKLEIK

SEQ ID NO: 7 - DNA, 354 bp, Artificial Sequence
  Nucleic acid sequence of murine anti-DR5-05 variable heavy chain
gaggtccagctgcagcagtctggggcagagcttgtgaagccaggggcctcagtcaagttgttctgcacagcttctggcttcaacattaaagacacccatatacactgggtgaaacagaggcctgagcagggcctggagtggattggaaggattgatcctgcgaatggtaatactgaatatgacccgaagttccagggcaaggccactataagagtagacacatcctccgacacagcctacctgcagctcagcagcctgacatctgaggacactgccgtccattattgtgctagatgggggactaacgtctattttgcttactggggtcaaggaacctcggtcaccgtctcctca

SEQ ID NO: 8 - protein, 118 aa, Artificial Sequence
  Amino acid sequence of murine anti-DR5-05 variable heavy chain
EVQLQQSGAELVKPGASVKLFCTASGFNIKDTHIHWVKQRPEQGLEWIGRIDPANGNTEYDPKFQGKATIRVDTSSDTAYLQLSSLTSEDTAVHYCARWGTNVYFAYWGQGTSVTVSS

SEQ ID NO: 9 - DNA, 993 bp, Artificial Sequence
  Nucleic acid sequence of human anti-DR5-01 or human anti-DR5-05 constant heavy chain
gcctccaccaagggcccatcggtcttccccctggcaccctcctccaagagcacctctgggggcacagcggccctgggctgcctggtcaaggactacttccccgaaccggtgacggtgtcgtggaactcaggcgccctgaccagcggcgtgcacaccttcccggctgtcctacagtcctcaggactctactccctcagcagcgtcgtgaccgtgccctccagcagcttgggcacccagacctacatctgcaacgtgaatcacaagcccagcaacaccaaggtggacaagaaagttgagcccaaatcttgtgacaaaactcacacatgcccaccgtgcccagcacctgaactcctggggggaccgtcagtcttcctcttccccccaaaacccaaggacaccctcatgatctcccggacccctgaggtcacatgcgtggtggtggacgtgagccacgaagaccctgaggtcaagttcaactggtacgtggacggcgtggaggtgcataatgccaagacaaagccgcgggaggagcagtacaacagcacgtaccgtgtggtcagcgtcctcaccgtcctgcaccaggactggctgaatggcaaggagtacaagtgcaaggtctccaacaaagccctcccagcccccatcgagaaaaccatctccaaagccaaagggcagccccgagaaccacaggtgtacaccctgcccccatcccgggatgagctgaccaagaaccaggtcagcctgacctgcctggtcaaaggcttctatcccagcgacatcgccgtggagtgggagagcaatgggcagccggagaacaactacaagaccacgcctcccgtgctggactccgacggctccttcttcctctacagcaagctcaccgtggacaagagcaggtggcagcaggggaacgtcttctcatgctccgtgatgcatgaggctctgcacaaccactacacgcagaagagcctctccctgtctccgggtaaatag

SEQ ID NO: 10 - protein, 330 aa, Artificial Sequence [sequence omitted]

SEQ ID NO: 11 - DNA, 324 bp, Artificial Sequence
  Nucleic acid sequence of human anti-DR5-01 or human anti-DR5-05 constant light chain
cgaactgtggctgcaccatctgtcttcatcttcccgccatctgatgagcagttgaaatctggaactgcctctgttgtgtgcctgctgaataacttctatcccagagaggccaaagtacagtggaaggtggataacgccctccaatcgggtaactcccaggagagtgtcacagagcaggacagcaaggacagcacctacagcctcagcagcaccctgacgctgagcaaagcagactacgagaaacacaaagtctacgcctgcgaagtcacccatcagggcctgagctcgcccgtcacaaagagcttcaacaggggagagtgttag

SEQ ID NO: 12 - protein, 107 aa, Artificial Sequence [sequence omitted]

SEQ ID NO: 13 - protein, 8 aa, Artificial Sequence
  murine anti-DR5-01 heavy chain CDR1 (IGMT numbering system)
GFNIKDTF

SEQ ID NO: 14 - protein, 8 aa, Artificial Sequence
  murine anti-DR5-01 or anti-DR5-05 heavy chain CDR2 (IGMT or Common numbering system)
IDPANGNT

SEQ ID NO: 15 - protein, 11 aa, Artificial Sequence
  murine anti-DR5-01 heavy chain CDR3 (IGMT numbering system)
VRGLYTYYFDY

SEQ ID NO: 16 - protein, 6 aa, Artificial Sequence
  murine anti-DR5-01 light chain CDR1 (IGMT or Common numbering system)
QSISNN

SEQ ID NO: 17 - protein, 9 aa, Artificial Sequence
  murine anti-DR5-01 light chain CDR3 (IGMT, Kabat or Common numbering system)
QQGNSWPYT

SEQ ID NO: 18 - protein, 8 aa, Artificial Sequence
  murine anti-DR5-05 heavy chain CDR1 (IGMT numbering system)
GFNIKDTH

SEQ ID NO: 19 - protein, 11 aa, Artificial Sequence
  murine anti-DR5-05 heavy chain CDR3 (IGMT numbering system)
ARWGTNVYFAY

SEQ ID NO: 20 - protein, 5 aa, Artificial Sequence
  murine anti-DR5-05 light chain CDR1 (IGMT or Common numbering system)
SSVSY

SEQ ID NO: 21 - protein, 9 aa, Artificial Sequence
  murine anti-DR5-05 light chain CDR3 (IGMT, Kabat or Common numbering system)
QQYHSYPPT

SEQ ID NO: 22 - protein, 5 aa, Artificial Sequence
  murine anti-DR5-01 heavy chain CDR1 (Kabat numbering system)
DTFIH

SEQ ID NO: 23 - protein, 17 aa, Artificial Sequence
  murine anti-DR5-01 heavy chain CDR2 (Kabat numbering system)
RIDPANGNTKYDPKFQG

SEQ ID NO: 24 - protein, 9 aa, Artificial Sequence
  murine anti-DR5-01 heavy chain CDR3 (Kabat or Common numbering system)
GLYTYYFDY

SEQ ID NO: 25 - protein, 11 aa, Artificial Sequence
  murine anti-DR5-01 light chain CDR1 (Kabat numbering system)
RASQSISNNLH

SEQ ID NO: 26 - protein, 7 aa, Artificial Sequence
  murine anti-DR5-01 light chain CDR2 (Kabat numbering system)
FASQSIS

SEQ ID NO: 27 - protein, 5 aa, Artificial Sequence
  murine anti-DR5-05 heavy chain CDR1 (Kabat numbering system)
DTHIH

SEQ ID NO: 28 - protein, 17 aa, Artificial Sequence
  murine anti-DR5-05 heavy chain CDR2 (Kabat numbering system)
RIDPANGNTEYDPKFQG

SEQ ID NO: 29 - protein, 9 aa, Artificial Sequence
  murine anti-DR5-05 heavy chain CDR3 (Kabat or Common numbering system)
WGTNVYFAY

SEQ ID NO: 30 - protein, 10 aa, Artificial Sequence
  murine anti-DR5-05 light chain CDR1 (Kabat numbering system)
SASSSVSYMY

SEQ ID NO: 31 - protein, 7 aa, Artificial Sequence
  murine anti-DR5-05 light chain CDR2 (Kabat numbering system)
RTSNLAS

SEQ ID NO: 32 - protein, 4 aa, Artificial Sequence
  murine anti-DR5-01 heavy chain CDR1 (Common numbering system)
KDTF

SEQ ID NO: 33 - protein, 4 aa, Artificial Sequence
  murine anti-DR5-05 heavy chain CDR1 (Common numbering system)
KDTH

SEQ ID NO: 34 - DNA, 354 bp, Artificial Sequence
  Nucleic acid sequence of humanized anti-DR5-01 variable heavy chain
gaggtgcaactgcagcaatcaggagcagaagtcgtaaagcccggtgcctccgttaaacttagctgcaaagcaagtgggtttaatatcaaagatacattcatccattgggtcaaacaggcaccaggccagggccttgaatggatcggtcgcatcgacccagctaacggaaacactaagtatgaccctaagttccagggaaaggctacaattacaacagatacatcctccaataccgcttacatggagctgtcttccttgcggtctgaggatactgctgtgtattactgtgtacgtgggctgtacacatattacttcgattattggggccaggggactcttgtaaccgtttcctcc

SEQ ID NO: 35 - protein, 118 aa, Artificial Sequence
  Amino acid sequence of humanized anti-DR5-01 variable heavy chain
EVQLQQSGAEVVKPGASVKLSCKASGFNIKDTFIHWVKQAPGQGLEWIGRIDPANGNTKYDPKFQGKATITTDTSSNTAYMELSSLRSEDTAVYYCVRGLYTYYFDYWGQGTLVTVSS

SEQ ID NO: 36 - DNA, 321 bp, Artificial Sequence
  Nucleic acid sequence of humanized anti-DR5-01 variable light chain
gagattgttatgacacagtcccctgctacattgagtgttagtccaggcgaaagagctacactgtcatgtagggcctctcagtctattagcaataacctgcactggtatcagcaaaagccaggtcaagcccccaggctgctgattaagtttgcatctcaaagtattacaggaatccctgctcggttcagcggctccgggagtggaaccgagtttacactcacaatctcaagcctccagtccgaagacttcgccgtatattactgtcagcagggcaactcttggccctacaccttcggtcagggaaccaagctggagatcaag

SEQ ID NO: 37 - protein, 107 aa, Artificial Sequence
  Amino acid sequence of humanized anti-DR5-01 variable light chain
EIVMTQSPATLSVSPGERATLSCRASQSISNNLHWYQQKPGQAPRLLIKFASQSITGIPARFSGSGSGTEFTLTISSLQSEDFAVYYCQQGNSWPYTFGQGTKLEIK

SEQ ID NO: 38 - DNA, 354 bp, Artificial Sequence
  Nucleic acid sequence of humanized anti-DR5-05 variable heavy chain
caagttcagttggtacaatcaggtgcagaagttaaaaagccaggggcatctgttaaagtgtcttgcaaggcctccggctttaatatcaaggacacacacatgcattgggtgcgccaggccccaggccagcgactggagtggattgggcgtattgaccccgccaacggcaacaccgagtatgaccagaagtttcagggccgtgtaaccatcaccgtcgatacctcagcatcaaccgcttacatggagctttcatctcttcggtccgaagacacagccgtctattactgcgctcgatggggaacaaacgtttactttgcatattggggtcagggtactctcgtcaccgtgagcagt

SEQ ID NO: 39 - protein, 118 aa, Artificial Sequence
  Amino acid sequence of humanized anti-DR5-05 variable heavy chain
QVQLVQSGAEVKKPGASVKVSCKASGFNIKDTHMHWVRQAPGQRLEWIGRIDPANGNTEYDQKFQGRVTITVDTSASTAYMELSSLRSEDTAVYYCARWGTNVYFAYWGQGTLVTVSS

SEQ ID NO: 40 - DNA, 318 bp, Artificial Sequence
  Nucleic acid sequence of humanized anti-DR5-05 variable light chain
gatattcaacttacacaatctccctcttctctctccgcttcagtaggggatagagtgaccatcacttgctctgcttcttccagcgtgtcatatatgtattggtatcagcaaaagcccggcaaggcacctaaaccatggatttacagaaccagcaatcttgccagcggtgttccaagtaggtttagcggctccggctctggtacagactttaccctgactatctcctctctccagcccgaggattttgccacatattactgccagcaataccattcttaccctccaacttttggaggtggcactaaggtggagatcaag

SEQ ID NO: 41 - protein, 106 aa, Artificial Sequence
  Amino acid sequence of humanized anti-DR5-05 variable light chain
DIQLTQSPSSLSASVGDRVTITCSASSSVSYMYWYQQKPGKAPKPWIYRTSNLASGVPSRFSGSGSGTDFTLTISSLQPEDFATYYCQQYHSYPPTFGGGTKVEIK